European Patent Specification EP 3 443 933 B1, published July 26, 2023. Title: Textured Surfaces for Breast Implants. Applicant: Establishment Labs S.A. Application EP18207556.4. The sequence listing filed with the application follows.

SEQUENCE LISTING (8 sequences)

SEQ ID NO: 1 - DNA, 21 bp, Artificial Sequence
  PCNA Primer Sequence Left
tggagaacttggaaatggaaa

SEQ ID NO: 2 - DNA, 24 bp, Artificial Sequence
  PCNA Primer Sequence Right
gaactggttcattcatctctatgg

SEQ ID NO: 3 - DNA, 19 bp, Artificial Sequence
  VCL Primer Sequence Left
ctgaaccaggccaaaggtt

SEQ ID NO: 4 - DNA, 20 bp, Artificial Sequence
  VCL Primer Sequence Right
gatctgtctgatggcctgct

SEQ ID NO: 5 - DNA, 20 bp, Artificial Sequence
  IL8 Primer Sequence Left
agacagcagagcacacaagc

SEQ ID NO: 6 - DNA, 18 bp, Artificial Sequence
  IL8 Primer Sequence Right
atggttccttccggtggt

SEQ ID NO: 7 - DNA, 20 bp, Artificial Sequence
  TNF-a Primer Sequence Left
agcccatgttgtagcaaacc

SEQ ID NO: 8 - DNA, 18 bp, Artificial Sequence
  TNF-a Primer Sequence Right
tctcagctccacgccatt